European Patent Specification EP 3 589 644 B1, published February 1, 2023. Title: Santalene Synthase. Applicant: Isobionics B.V. The sequence listing filed with the application follows.

SEQUENCE LISTING (33 sequences)

SEQ ID NO: 1 - DNA, 1662 bp, Cinnamomum camphora
atggactccatggaggtacgccgctctgcaatctatcactcgaccttttgggatattgatagcattcgcgccctgctcgcaagaagagactgcactgctgcagctgcattgagtcctgaccatcacaaaagactcaaggaaagaattcagcgccggctacaagacatcacacagccacaccatctgcttggattgatcgacgctgtccaacgcctcggtgtggcctaccagtttgaggaagaaatcagtgacgcactgcatgggcttcactcagagaacacggagcatgcaattaaggacagtctgcaccacacatctctctattttagattgcttaggcaacatgggtgtaacctttcatcagacatattcaacaaatttaagaaggaaggaggaggtttcaaggcaagcctatgtgaggatgcaatgggacttttgagcttgtatgaggctgtacgtcttagcgtcaaaggtgaagccatcttggaggaagctcaggtcttctcgatcgcgaatttgaagattctgatggaaagggtggagaggaagctggcagatagaatagaacatgccttggagatccccttgtattggagggcgccgagactggaagctagatggtacatagatgtatatgaaaaggaagatgggaggattgatgacttgcttgattttgcaaagctagatttcaacagggtgcaaatgttgtaccaaaccgaactgaaggaattatcaatgtggtgggaattgctggggttaccagcgaagatggggttcttccgagacagactattggagaaccatctcttttcaattgcagtggttgtcgagcctcaatactcccagtgtagagtagcaattacaaaagccatagtccttatgacagcaatggatgacttttatgatgtgcatggtttgccagatgagctaaaagtcttcacggacaccgttaatcggtgggatttagagggaattgatcaactaccagagtatatgaagctgtactacttggcgttatataatacaaccaatgagaccgcatacatcatcctcaaggagaagggattcaatgctacacattatctgaagaaactgtgggcaatgcaaagtaacgcgtactttcgggaagctcaatggttcaacagtggttacatacctaaatttgatgagtatttagacaatgctttagtctcagttggggcgccctttgtattgggtctctcataccccatgatacaacaacaaatatcaaaggaggaaattgatttaatccccgaagatctaaatctcctccgttgggcatcgatcatatttcgactatatgatgatttggccacttcaaaggctgagcaacaacgtggggacgtgccaaaatccatccaatgttatatgcatgaaactggtagttcggaggaagttgcagcaaaccatatcagggacctcatcagtgatgcttggaaggaagtgaatgcagagtgtttgaaacctacttctctgtcaaagcattacgtgggagtagctccaaattcggctaggtctggagtgctgatgtaccatcatgactttgatggctttgcaagtccccatggcaggactaatgctcatatcacgtcaatattttttgaaccagtgccattgaaggaatccatcaacttgggatga

SEQ ID NO: 2 - DNA, 1758 bp, artificial sequence
  codon optimized sequence
aaatcataaaaaatttatttgctttgtgagcggataacaattattagattcaccggcgagccagcaggaatttcacttagatgacaggagggacatatggacagcatggaagtccggcggtcggcgatctaccacagcacgttctgggacatcgacagcatccgggcgctcctggcgcggcgggactgcacggcggccgcggccctctcgcccgaccaccataagcgcctgaaggagcgcatccagcgccgcctccaggacatcacccagccccaccatctgctcggcctcatcgacgccgtgcagcgcctgggcgtggcctaccagttcgaggaagagatctcggacgcgctgcacggcctccattcggagaacaccgagcacgccatcaaggactcgctgcaccatacgtcgctctatttccgcctgctccgccagcatggctgcaacctgtcgtcggacatcttcaacaagttcaagaaggaaggcggcggcttcaaggcctcgctctgcgaggacgccatgggcctgctctcgctgtatgaggccgtgcgcctctcggtgaagggcgaggccatcctggaggaagcccaggtgttctcgatcgccaacctgaagatcctcatggagcgcgtggagcgcaagctcgccgaccgcatcgagcatgccctggagatcccgctctattggcgcgccccgcgtctggaggcccgctggtacatcgacgtgtatgagaaggaagacggccgcatcgacgacctgctcgacttcgcgaagctggacttcaaccgcgtgcagatgctctatcagaccgagctgaaggagctctcgatgtggtgggagctgctgggcctgcccgccaagatgggcttcttccgcgaccgcctgctcgagaaccacctcttctcgatcgccgtggtggtggagccccagtactcgcagtgccgcgtggccatcaccaaggcgatcgtgctgatgacggcgatggacgacttctatgacgtgcatggcctgccggacgagctcaaggtgttcaccgacacggtgaaccgctgggacctggagggcatcgaccagctccccgagtacatgaagctgtactatctggcgctctacaacaccacgaacgagacggcctatatcatcctgaaggagaagggcttcaacgccacgcattacctgaagaagctctgggccatgcagtcgaacgcgtatttccgcgaggcccagtggttcaactcgggctacatcccgaagttcgacgagtatctggacaacgccctcgtgtcggtgggcgccccgttcgtgctgggcctctcgtatcccatgatccagcagcagatctcgaaggaagagatcgacctgatccccgaggacctcaacctgctccgctgggcctcgatcatcttccgcctgtacgacgacctggccacctcgaaggccgagcagcagcgcggcgacgtgcccaagtcgatccagtgctatatgcatgagacgggctcgtcggaggaagtggcggccaaccatatccgcgacctgatctcggacgcgtggaaggaagtgaacgccgagtgcctgaagccgacctcgctctcgaagcactacgtgggcgtggcccccaactcggcccgctcgggcgtgctcatgtatcaccatgacttcgacggcttcgcgtcgccccatggccgcacgaacgcccacatcacgagcatcttcttcgagccggtccccctcaaggagagcatcaacctgggctga

SEQ ID NO: 3 - protein, 553 aa, Cinnamomum camphora
MDSMEVRRSAIYHSTFWDIDSIRALLARRDCTAAAALSPDHHKRLKERIQRRLQDITQPHHLLGLIDAVQRLGVAYQFEEEISDALHGLHSENTEHAIKDSLHHTSLYFRLLRQHGCNLSSDIFNKFKKEGGGFKASLCEDAMGLLSLYEAVRLSVKGEAILEEAQVFSIANLKILMERVERKLADRIEHALEIPLYWRAPRLEARWYIDVYEKEDGRIDDLLDFAKLDFNRVQMLYQTELKELSMWWELLGLPAKMGFFRDRLLENHLFSIAVVVEPQYSQCRVAITKAIVLMTAMDDFYDVHGLPDELKVFTDTVNRWDLEGIDQLPEYMKLYYLALYNTTNETAYIILKEKGFNATHYLKKLWAMQSNAYFREAQWFNSGYIPKFDEYLDNALVSVGAPFVLGLSYPMIQQQISKEEIDLIPEDLNLLRWASIIFRLYDDLATSKAEQQRGDVPKSIQCYMHETGSSEEVAANHIRDLISDAWKEVNAECLKPTSLSKHYVGVAPNSARSGVLMYHHDFDGFASPHGRTNAHITSIFFEPVPLKESINLG

SEQ ID NO: 4 - DNA, 2636 bp, artificial sequence
  SPppa-MBP-CiCaSSy
aaatttatttgctttgtgagcggataacaattattagattcaccggcgagccagcaggaatttcactctagatgacaggagggacatcatacgacgacgacaagatcttccaggacaagctctatcccttcacgtgggacgccgtgcgctacaacggcaagctgatcgcgtatcccatcgcggtggaggccctgtcgctcatctataacaaggacctgctcccgaacccgcccaagacctgggaggagatccccgccctcgacaaggagctgaaggccaagggcaagtcggcgctcatgttcaacctgcaggagccgtacttcacctggcccctgatcgcggccgacggcggctacgcgttcaagtatgagaacggcaagtatgacatcaaggacgtgggcgtggacaacgcgggcgccaaggccggcctgaccttcctcgtggacctgatcaagaacaagcacatgaacgccgacacggactactcgatcgcggaggccgcgttcaacaagggcgagaccgccatgacgatcaacggcccgtgggcgtggtcgaacatcgacacctcgaaggtgaactatggcgtgaccgtgctccccacgttcaagggccagccctcgaagcccttcgtgggcgtgctgtcggcgggcatcaacgccgcgtcgccgaacaaggagctcgcgaaggagttcctggagaactacctgctcaccgacgagggcctggaggccgtgaacaaggacaagcccctgggcgccgtggccctgaagtcgtatgaggaagagctggtgaaggacccgcgcatcgcggccaccatggagaacgcgcagaagggcgagatcatgccgaacatcccccagatgtcggccttctggtatgcggtgcgcaccgccgtgatcaacgcggcctcgggccgccagaccgtggacgaggccctcaaggacgcccagaccggcgacgacgacgacaagatcatggacagcatggaagtccggcggtcggcgatctaccacagcacgttctgggacatcgacagcatccgggcgctcctggcgcggcgggactgcacggcggccgcggccctctcgcccgaccaccataagcgcctgaaggagcgcatccagcgccgcctccaggacatcacccagccccaccatctgctcggcctcatcgacgccgtgcagcgcctgggcgtggcctaccagttcgaggaagagatctcggacgcgctgcacggcctccattcggagaacaccgagcacgccatcaaggactcgctgcaccatacgtcgctctatttccgcctgctccgccagcatggctgcaacctgtcgtcggacatcttcaacaagttcaagaaggaaggcggcggcttcaaggcctcgctctgcgaggacgccatgggcctgctctcgctgtatgaggccgtgcgcctctcggtgaagggcgaggccatcctggaggaagcccaggtgttctcgatcgccaacctgaagatcctcatggagcgcgtggagcgcaagctcgccgaccgcatcgagcatgccctggagatcccgctctattggcgcgccccgcgtctggaggcccgctggtacatcgacgtgtatgagaaggaagacggccgcatcgacgacctgctcgacttcgcgaagctggacttcaaccgcgtgcagatgctctatcagaccgagctgaaggagctctcgatgtggtgggagctgctgggcctgcccgccaagatgggcttcttccgcgaccgcctgctcgagaaccacctcttctcgatcgccgtggtggtggagccccagtactcgcagtgccgcgtggccatcaccaaggcgatcgtgctgatgacggcgatggacgacttctatgacgtgcatggcctgccggacgagctcaaggtgttcaccgacacggtgaaccgctgggacctggagggcatcgaccagctccccgagtacatgaagctgtactatctggcgctctacaacaccacgaacgagacggcctatatcatcctgaaggagaagggcttcaacgccacgcattacctgaagaagctctgggccatgcagtcgaacgcgtatttccgcgaggcccagtggttcaactcgggctacatcccgaagttcgacgagtatctggacaacgccctcgtgtcggtgggcgccccgttcgtgctgggcctctcgtatcccatgatccagcagcagatctcgaaggaagagatcgacctgatccccgaggacctcaacctgctccgctgggcctcgatcatcttccgcctgtacgacgacctggccacctcgaaggccgagcagcagcgcggcgacgtgcccaagtcgatccagtgctatatgcatgagacgggctcgtcggaggaagtggcggccaaccatatccgcgacctgatctcggacgcgtggaaggaagtgaacgccgagtgcctgaagccgacctcgctctcgaagcactacgtgggcgtggcccccaactcggcccgctcgggcgtgctcatgtatcaccatgacttcgacggcttcgcgtcgccccatggccgcacgaacgcccacatcacgagcatcttcttcgagccggtccccctcaaggagagcatcaacctgggctga

SEQ ID NO: 5 - protein, 927 aa, artificial protein
  MBP-CiCaSSy
MKIEEGKLVIWINGDKGYNGLAEVGKKFEKDTGIKVTVEHPDKLEEKFPQVAATGDGPDIIFWAHDRFGGYAQSGLLAEITPDKAFQDKLYPFTWDAVRYNGKLIAYPIAVEALSLIYNKDLLPNPPKTWEEIPALDKELKAKGKSALMFNLQEPYFTWPLIAADGGYAFKYENGKYDIKDVGVDNAGAKAGLTFLVDLIKNKHMNADTDYSIAEAAFNKGETAMTINGPWAWSNIDTSKVNYGVTVLPTFKGQPSKPFVGVLSAGINAASPNKELAKEFLENYLLTDEGLEAVNKDKPLGAVALKSYEEELVKDPRIAATMENAQKGEIMPNIPQMSAFWYAVRTAVINAASGRQTVDEALKDAQTGDDDDKIMDSMEVRRSAIYHSTFWDIDSIRALLARRDCTAAAALSPDHHKRLKERIQRRLQDITQPHHLLGLIDAVQRLGVAYQFEEEISDALHGLHSENTEHAIKDSLHHTSLYFRLLRQHGCNLSSDIFNKFKKEGGGFKASLCEDAMGLLSLYEAVRLSVKGEAILEEAQVFSIANLKILMERVERKLADRIEHALEIPLYWRAPRLEARWYIDVYEKEDGRIDDLLDFAKLDFNRVQMLYQTELKELSMWWELLGLPAKMGFFRDRLLENHLFSIAVVVEPQYSQCRVAITKAIVLMTAMDDFYDVHGLPDELKVFTDTVNRWDLEGIDQLPEYMKLYYLALYNTTNETAYIILKEKGFNATHYLKKLWAMQSNAYFREAQWFNSGYIPKFDEYLDNALVSVGAPFVLGLSYPMIQQQISKEEIDLIPEDLNLLRWASIIFRLYDDLATSKAEQQRGDVPKSIQCYMHETGSSEEVAANHIRDLISDAWKEVNAECLKPTSLSKHYVGVAPNSARSGVLMYHHDFDGFASPHGRTNAHITSIFFEPVPLKESINLG

SEQ ID NO: 6 - DNA, 2282 bp, artificial sequence
  PcrtE-TRX-CiCaSSy
cgctgctgaacgcgatggcggcgcggggcgcgacgcgcggggccgcatccgtctgcatcggcgggggcgaggcgacggccatcgcgctggaacggctgagctaattcatttgcgcgaatccgcgtttttcgtgcacgatgggggaaccggaaacggccacgcctgttgtggttgcgtcgacctgtcttcgggccatgcccgtgacgcgatgtggcaggcgcatggggcgttgccgatccggtcgcatgactgacgcaacgaaggcacatatgtcggacaagatcatccacctgaccgacgacagcttcgacaccgacgtgctgaaggccgacggcgccatcctcgtcgatttctgggccgaatggtgcggcccctgcaagatgatcgcgccgatcctcgacgagatcgccgacgaatatcagggcaagctgaccgtcgccaagctgaacatcgaccagaacccgggcacggcgccgaaatacggcatccgcggcatcccgacgctgctgctcttcaagaacggcgaggtggcggccaccaaggtcggcgcgctgtcgaagggccagctgaaggagttcctcgatgcgaacctcgccggtggtgatgacgacgacaagattatggacagcatggaagtccggcggtcggcgatctaccacagcacgttctgggacatcgacagcatccgggcgctcctggcgcggcgggactgcacggcggccgcggccctctcgcccgaccaccataagcgcctgaaggagcgcatccagcgccgcctccaggacatcacccagccccaccatctgctcggcctcatcgacgccgtgcagcgcctgggcgtggcctaccagttcgaggaagagatctcggacgcgctgcacggcctccattcggagaacaccgagcacgccatcaaggactcgctgcaccatacgtcgctctatttccgcctgctccgccagcatggctgcaacctgtcgtcggacatcttcaacaagttcaagaaggaaggcggcggcttcaaggcctcgctctgcgaggacgccatgggcctgctctcgctgtatgaggccgtgcgcctctcggtgaagggcgaggccatcctggaggaagcccaggtgttctcgatcgccaacctgaagatcctcatggagcgcgtggagcgcaagctcgccgaccgcatcgagcatgccctggagatcccgctctattggcgcgccccgcgtctggaggcccgctggtacatcgacgtgtatgagaaggaagacggccgcatcgacgacctgctcgacttcgcgaagctggacttcaaccgcgtgcagatgctctatcagaccgagctgaaggagctctcgatgtggtgggagctgctgggcctgcccgccaagatgggcttcttccgcgaccgcctgctcgagaaccacctcttctcgatcgccgtggtggtggagccccagtactcgcagtgccgcgtggccatcaccaaggcgatcgtgctgatgacggcgatggacgacttctatgacgtgcatggcctgccggacgagctcaaggtgttcaccgacacggtgaaccgctgggacctggagggcatcgaccagctccccgagtacatgaagctgtactatctggcgctctacaacaccacgaacgagacggcctatatcatcctgaaggagaagggcttcaacgccacgcattacctgaagaagctctgggccatgcagtcgaacgcgtatttccgcgaggcccagtggttcaactcgggctacatcccgaagttcgacgagtatctggacaacgccctcgtgtcggtgggcgccccgttcgtgctgggcctctcgtatcccatgatccagcagcagatctcgaaggaagagatcgacctgatccccgaggacctcaacctgctccgctgggcctcgatcatcttccgcctgtacgacgacctggccacctcgaaggccgagcagcagcgcggcgacgtgcccaagtcgatccagtgctatatgcatgagacgggctcgtcggaggaagtggcggccaaccatatccgcgacctgatctcggacgcgtggaaggaagtgaacgccgagtgcctgaagccgacctcgctctcgaagcactacgtgggcgtggcccccaactcggcccgctcgggcgtgctcatgtatcaccatgacttcgacggcttcgcgtcgccccatggccgcacgaacgcccacatcacgagcatcttcttcgagccggtccccctcaaggagagcatcaacctgggctga

SEQ ID NO: 7 - protein, 670 aa, artificial sequence
  TRX-CiCaSSy
MSDKIIHLTDDSFDTDVLKADGAILVDFWAEWCGPCKMIAPILDEIADEYQGKLTVAKLNIDQNPGTAPKYGIRGIPTLLLFKNGEVAATKVGALSKGQLKEFLDANLAGGDDDDKIMDSMEVRRSAIYHSTFWDIDSIRALLARRDCTAAAALSPDHHKRLKERIQRRLQDITQPHHLLGLIDAVQRLGVAYQFEEEISDALHGLHSENTEHAIKDSLHHTSLYFRLLRQHGCNLSSDIFNKFKKEGGGFKASLCEDAMGLLSLYEAVRLSVKGEAILEEAQVFSIANLKILMERVERKLADRIEHALEIPLYWRAPRLEARWYIDVYEKEDGRIDDLLDFAKLDFNRVQMLYQTELKELSMWWELLGLPAKMGFFRDRLLENHLFSIAVVVEPQYSQCRVAITKAIVLMTAMDDFYDVHGLPDELKVFTDTVNRWDLEGIDQLPEYMKLYYLALYNTTNETAYIILKEKGFNATHYLKKLWAMQSNAYFREAQWFNSGYIPKFDEYLDNALVSVGAPFVLGLSYPMIQQQISKEEIDLIPEDLNLLRWASIIFRLYDDLATSKAEQQRGDVPKSIQCYMHETGSSEEVAANHIRDLISDAWKEVNAECLKPTSLSKHYVGVAPNSARSGVLMYHHDFDGFASPHGRTNAHITSIFFEPVPLKESINLG

SEQ ID NO: 8 - DNA, 39 bp, artificial sequence
  primer
atatggatcctatggactccatggaggtacgccgctctg

SEQ ID NO: 9 - DNA, 47 bp, artificial sequence
  TS23 RE
atatgcggccgctcatcccaagttgatggattccttcaatggcactg

SEQ ID NO: 10 - protein, 553 aa, artificial sequence
  TS23-1
MDSMEVRRSANYHSTFWDIDSIRALLARRDCTVAAALSHDHHKRLKERIQRRLQDITQPHHLLGLIDAVQRLGVAYQFEEEISDALHGLHSENTEHAIKDSLHHTSLYFRLLRQHGCNLSSDIFNKFKKEGGGFKASLCEDAMGLLSLYEAAHLGVKSEAILEEAQVFSTSNLKILMERVERKLADRIDHALEIPLYWRAPRVEARWYIDVYEKEDGRIDDLLDFAKLDFNRVQMLYQTELKELSMWWELLGLPEKMGFFRDRLLESHLFSIGVVVEPQYSQCRVAITKALVLFTAMDDFYDVHGLPEELKVFTDTVNRWDLEGIDQLPEYMKLYYLALYNTTNETAYIILKEKGFNATHYLKKLWAMQSNSYFREAQWFNSGYIPKFDEYLDNALVSVGVPLLLGLSYPMIQQHISKAEIDLIPEDLNLLRWASIIFRLYNDLATSKAEQQRGDVPKSIQCYMHETGSSEEVAANHIRDLISDAWKELNAECLKPTSLSKHYVGVAPNSARSGVLMYHHDFDGFASPHSRTNAHITSIFFEPVPLKESINLG

SEQ ID NO: 11 - protein, 553 aa, artificial sequence
  TS23-2
MDSMEVRRSANYHSTFWDIDSIRALLARRDCTVAAALSHDHHKRLKERIQRRLQDITQPHHLLGLIDAVQRLGVAYQFEEEISDALHGLHSENTEHAVKDSLHHTSLYFRLLRQHGCNLSTDIFNKFKKEGGGFKASLCEDAMGLLSLYEAAHLGVKSEAILEEAQVFSTSNLKILMERVERKLADRIDHALEIPLYWRAPRVEARWYIDVYEKEDGRIDDLLDFAKLDFNRVQMLYQTELKELSMWWELLGLPEKMGFFRDRLLESHLFSIGVVVEPQYSQCRVAITKALVLFTAMDDFYDVHGLPEELKVFTDTVNRWDLEGIDQLPEYMKLYYLALYNTTNETAYIILKEKGFNATHYLKKLWAMQSNSYFREAQWFNSGYIPKFDEYLDNALVSVGVPLLLGLSYPMIQQHISKAEIDLIPEDLNLLRWASIIFRLYNDLATSKAEQQRGDVPKSIQCYMHETGSSEEVAANHIRDLISDAWKEVNAECLKPTSLSKHYVGVAPNSARSGVLMYHHDFDGFASPHSRTNAHITSIFFEPVPLKESINLG

SEQ ID NO: 12 - DNA, 21 bp, artificial sequence
  primer
gctgttagcgggcccattaag

SEQ ID NO: 13 - DNA, 40 bp, artificial sequence
  primer
gatattctcattttagccattttagcttccttagctcctg

SEQ ID NO: 14 - DNA, 40 bp, artificial sequence
  primer
caggagctaaggaagctaaaatggctaaaatgagaatatc

SEQ ID NO: 15 - DNA, 39 bp, artificial sequence
  primer
ccaagcgagctcgatatcaaactaaaacaattcatccag

SEQ ID NO: 16 - DNA, 23 bp, artificial sequence
  primer
ctgtccatgatcttgtcgtcgtc

SEQ ID NO: 17 - DNA, 44 bp, artificial sequence
  primer
actggcctcagaattcaaatttatttgctttgtgagcggataac

SEQ ID NO: 18 - DNA, 25 bp, artificial sequence
  primer
caagatcatggacagcatggaagtc

SEQ ID NO: 19 - DNA, 28 bp, artificial sequence
  primer
tttatgatttggatcctcagcccaggtt

SEQ ID NO: 20 - DNA, 25 bp, artificial sequence
  primer
ctgtccataatcttgtcgtcgtcat

SEQ ID NO: 21 - DNA, 28 bp, artificial sequence
  primer
actggcctcagaattccgctgctgaacg

SEQ ID NO: 22 - DNA, 26 bp, artificial
  primer
caagattatggacagcatggaagtcc

SEQ ID NO: 23 - DNA, 28 bp, artificial
  primer
tttatgatttggatcctcagcccaggtt

SEQ ID NO: 24 - DNA, 2330 bp, artificial
  PcrtE-TRX-SaSSy
cgctgctgaacgcgatggcggcgcggggcgcgacgcgcggggccgcatccgtctgcatcggcgggggcgaggcgacggccatcgcgctggaacggctgagctaattcatttgcgcgaatccgcgtttttcgtgcacgatgggggaaccggaaacggccacgcctgttgtggttgcgtcgacctgtcttcgggccatgcccgtgacgcgatgtggcaggcgcatggggcgttgccgatccggtcgcatgactgacgcaacgaaggcacatatgtcggacaagatcatccacctgaccgacgacagcttcgacaccgacgtgctgaaggccgacggcgccatcctcgtcgatttctgggccgaatggtgcggcccctgcaagatgatcgcgccgatcctcgacgagatcgccgacgaatatcagggcaagctgaccgtcgccaagctgaacatcgaccagaacccgggcacggcgccgaaatacggcatccgcggcatcccgacgctgctgctcttcaagaacggcgaggtggcggccaccaaggtcggcgcgctgtcgaagggccagctgaaggagttcctcgatgcgaacctcgccggtggtgatgacgacgacaagattatggacagcagcaccgcgaccgccatgaccgcccccttcatcgaccccaccgaccacgtgaacctcaagaccgacaccgacgccagcgagaaccgtcgcatgggcaactacaagccgtcgatctggaactatgacttcctgcagagcctcgccacccaccataacatcgtggaggagcgccacctcaagctggcggagaagctgaagggccaggtcaagttcatgttcggcgcccctatggagcccctcgcgaagctcgagctggtcgacgtggtccagcggctcggcctgaaccacctgttcgagaccgagatcaaggaagccctcttctcgatctacaaggacggcagcaacgggtggtggttcggccacctgcatgcgacgtcgctccgcttccggctgctccgccagtgcggcctgttcatcccccaggacgtgttcaagaccttccagaacaagacgggcgagttcgacatgaagctctgcgacaacgtcaagggcctgctctcgctgtacgaggccagctatctcggctggaagggcgagaacatcctggacgaggccaaggcgttcaccacgaagtgcctcaagtcggcctgggagaacatcagcgagaagtggctggcgaagcgcgtgaagcacgccctcgcgctgccgctccattggcgcgtcccccggatcgaggcgcggtggttcatcgaggcctatgagcaggaagccaacatgaacccgaccctgctcaagctggccaagctcgacttcaacatggtgcagtcgatccaccagaaggagatcggcgagctggcgcggtggtgggtcaccacgggcctggacaagctcgccttcgcgcggaacaacctgctccagtcgtacatgtggagctgcgccatcgcgtcggaccccaagttcaagctggcccgcgagaccatcgtggagatcggctcggtcctcacggtggtcgacgacggctacgacgtgtatggcagcatcgacgagctggacctctatacctcgagcgtggagcggtggtcgtgcgtcgagatcgacaagctcccgaacaccctgaagctcatcttcatgtcgatgttcaacaagacgaacgaggtcggcctccgcgtccagcatgagcggggctacaactcgatccccacgttcatcaaggcctgggtggagcagtgcaagtcgtatcagaaggaagcccgctggttccacggtggccataccccgcccctggaggagtactcgctgaacggcctcgtgagcatcggcttcccgctgctcctgatcacgggctatgtggccatcgcggagaacgaggccgcgctggacaaggtccacccgctccccgacctgctgcattactcgagcctcctgtcgcgcctgatcaacgacatcggcaccagccccgacgagatggcgcggggcgacaacctcaagtcgatccactgctatatgaacgagacgggcgccagcgaggaagtggcgcgcgagcatatcaagggcgtcatcgaggagaactggaagatcctgaaccagtgctgcttcgaccagtcgcagttccaggagccgttcatcaccttcaacctcaactcggtgcgcggcagccacttcttctacgagttcggcgacggcttcggcgtcacggactcgtggacgaaggtggacatgaagagcgtgctgatcgaccccatccccctgggcgaggagtga

SEQ ID NO: 25 - protein, 686 aa, artificial
  TRX-SaSSy
MSDKIIHLTDDSFDTDVLKADGAILVDFWAEWCGPCKMIAPILDEIADEYQGKLTVAKLNIDQNPGTAPKYGIRGIPTLLLFKNGEVAATKVGALSKGQLKEFLDANLAGGDDDDKIMDSSTATAMTAPFIDPTDHVNLKTDTDASENRRMGNYKPSIWNYDFLQSLATHHNIVEERHLKLAEKLKGQVKFMFGAPMEPLAKLELVDVVQRLGLNHLFETEIKEALFSIYKDGSNGWWFGHLHATSLRFRLLRQCGLFIPQDVFKTFQNKTGEFDMKLCDNVKGLLSLYEASYLGWKGENILDEAKAFTTKCLKSAWENISEKWLAKRVKHALALPLHWRVPRIEARWFIEAYEQEANMNPTLLKLAKLDFNMVQSIHQKEIGELARWWVTTGLDKLAFARNNLLQSYMWSCAIASDPKFKLARETIVEIGSVLTVVDDGYDVYGSIDELDLYTSSVERWSCVEIDKLPNTLKLIFMSMFNKTNEVGLRVQHERGYNSIPTFIKAWVEQCKSYQKEARWFHGGHTPPLEEYSLNGLVSIGFPLLLITGYVAIAENEAALDKVHPLPDLLHYSSLLSRLINDIGTSPDEMARGDNLKSIHCYMNETGASEEVAREHIKGVIEENWKILNQCCFDQSQFQEPFITFNLNSVRGSHFFYEFGDGFGVTDSWTKVDMKSVLIDPIPLGEE

SEQ ID NO: 26 - protein, 495 aa, artificial [sequence omitted]

SEQ ID NO: 27 - protein, 117 aa, artificial
  TRX
MSDKIIHLTDDSFDTDVLKADGAILVDFWAEWCGPCKMIAPILDEIADEYQGKLTVAKLNIDQNPGTAPKYGIRGIPTLLLFKNGEVAATKVGALSKGQLKEFLDANLAGGDDDDKI

SEQ ID NO: 28 - protein, 374 aa, artificial
  MBP
MKIEEGKLVIWINGDKGYNGLAEVGKKFEKDTGIKVTVEHPDKLEEKFPQVAATGDGPDIIFWAHDRFGGYAQSGLLAEITPDKAFQDKLYPFTWDAVRYNGKLIAYPIAVEALSLIYNKDLLPNPPKTWEEIPALDKELKAKGKSALMFNLQEPYFTWPLIAADGGYAFKYENGKYDIKDVGVDNAGAKAGLTFLVDLIKNKHMNADTDYSIAEAAFNKGETAMTINGPWAWSNIDTSKVNYGVTVLPTFKGQPSKPFVGVLSAGINAASPNKELAKEFLENYLLTDEGLEAVNKDKPLGAVALKSYEEELVKDPRIAATMENAQKGEIMPNIPQMSAFWYAVRTAVINAASGRQTVDEALKDAQTGDDDDKI

SEQ ID NO: 29 - protein, 40 aa, artificial
  SET
EEASVTSTEETLTPAQEAARTRAANKARKEAELAAATAEQ

SEQ ID NO: 30 - DNA, 3147 bp, artificial
  NusA-CiCaSSy
atgaacaaggagatcctcgcggtggtggaggcggtgtcgaacgagaaggcgctgccccgcgagaagatcttcgaggccctggagtcggccctggccaccgcgaccaagaagaagtacgagcaggagatcgacgtgcgcgtgcagatcgaccgcaagtcgggcgacttcgacacgttccgccgctggctcgtggtggacgaggtgacccagcccacgaaggagatcaccctggaggcggcccgctatgaggacgagtcgctgaacctcggcgactatgtggaggaccagatcgagtcggtgaccttcgaccgcatcaccacgcagacggcgaagcaggtgatcgtgcagaaggtgcgcgaggccgagcgcgccatggtggtggaccagttccgcgagcacgagggcgagatcatcaccggcgtggtgaagaaggtgaaccgcgacaacatctcgctggacctgggcaacaacgcggaggccgtgatcctgcgcgaggacatgctcccgcgcgagaacttccgcccgggcgaccgcgtgcgcggcgtgctctattcggtgcgccccgaggcccgtggcgcccagctgttcgtgacccgctcgaagccggagatgctgatcgagctcttccgcatcgaggtgcccgagatcggcgaggaagtgatcgagatcaaggcggccgcccgcgacccgggctcgcgcgcgaagatcgccgtgaagaccaacgacaagcgcatcgaccccgtgggcgcctgcgtgggcatgcgtggcgcccgcgtgcaggccgtgtcgaccgagctcggcggcgagcgcatcgacatcgtgctgtgggacgacaacccggcgcagttcgtgatcaacgccatggccccggcggacgtggcctcgatcgtggtggacgaggacaagcataccatggacatcgccgtggaggcgggcaacctggcccaggccatcggccgcaacggccagaacgtgcgcctggcctcgcagctctcgggctgggagctgaacgtgatgacggtggacgacctgcaggccaagcatcaggccgaggcccatgccgccatcgacaccttcacgaagtacctcgacatcgacgaggacttcgcgaccgtgctcgtggaggaaggcttctcgacgctggaggagctcgcctatgtgccgatgaaggagctgctcgagatcgagggcctggacgagccgacggtggaggcgctccgcgagcgcgccaagaacgccctggccaccatcgcccaggcccaggaagagtcgctgggcgacaacaagccggccgacgacctgctcaacctggagggcgtggaccgcgacctggccttcaagctcgccgcccgcggcgtgtgcacgctcgaggacctggccgagcagggcatcgacgacctggccgacatcgagggcctcaccgacgagaaggccggcgccctgatcatggccgcccgcaacatctgctggttcggcgacgaggcgatggacagcatggaagtccggcggtcggcgatctaccacagcacgttctgggacatcgacagcatccgggcgctcctggcgcggcgggactgcacggcggccgcggccctctcgcccgaccaccataagcgcctgaaggagcgcatccagcgccgcctccaggacatcacccagccccaccatctgctcggcctcatcgacgccgtgcagcgcctgggcgtggcctaccagttcgaggaagagatctcggacgcgctgcacggcctccattcggagaacaccgagcacgccatcaaggactcgctgcaccatacgtcgctctatttccgcctgctccgccagcatggctgcaacctgtcgtcggacatcttcaacaagttcaagaaggaaggcggcggcttcaaggcctcgctctgcgaggacgccatgggcctgctctcgctgtatgaggccgtgcgcctctcggtgaagggcgaggccatcctggaggaagcccaggtgttctcgatcgccaacctgaagatcctcatggagcgcgtggagcgcaagctcgccgaccgcatcgagcatgccctggagatcccgctctattggcgcgccccgcgtctggaggcccgctggtacatcgacgtgtatgagaaggaagacggccgcatcgacgacctgctcgacttcgcgaagctggacttcaaccgcgtgcagatgctctatcagaccgagctgaaggagctctcgatgtggtgggagctgctgggcctgcccgccaagatgggcttcttccgcgaccgcctgctcgagaaccacctcttctcgatcgccgtggtggtggagccccagtactcgcagtgccgcgtggccatcaccaaggcgatcgtgctgatgacggcgatggacgacttctatgacgtgcatggcctgccggacgagctcaaggtgttcaccgacacggtgaaccgctgggacctggagggcatcgaccagctccccgagtacatgaagctgtactatctggcgctctacaacaccacgaacgagacggcctatatcatcctgaaggagaagggcttcaacgccacgcattacctgaagaagctctgggccatgcagtcgaacgcgtatttccgcgaggcccagtggttcaactcgggctacatcccgaagttcgacgagtatctggacaacgccctcgtgtcggtgggcgccccgttcgtgctgggcctctcgtatcccatgatccagcagcagatctcgaaggaagagatcgacctgatccccgaggacctcaacctgctccgctgggcctcgatcatcttccgcctgtacgacgacctggccacctcgaaggccgagcagcagcgcggcgacgtgcccaagtcgatccagtgctatatgcatgagacgggctcgtcggaggaagtggcggccaaccatatccgcgacctgatctcggacgcgtggaaggaagtgaacgccgagtgcctgaagccgacctcgctctcgaagcactacgtgggcgtggcccccaactcggcccgctcgggcgtgctcatgtatcaccatgacttcgacggcttcgcgtcgccccatggccgcacgaacgcccacatcacgagcatcttcttcgagccggtccccctcaaggagagcatcaacctgggctga

SEQ ID NO: 31 - DNA, 1791 bp, artificial
  SET-CiCaSSy
atggaggaggccagcgtgaccagcaccgaggagaccctgaccccggcccaggaggccgcccgcacccgcgccgccaacaaggcccgcaaggaggccgagctggccgccgccaccgccgagcaggccgccatggacagcatggaagtccggcggtcggcgatctaccacagcacgttctgggacatcgacagcatccgggcgctcctggcgcggcgggactgcacggcggccgcggccctctcgcccgaccaccataagcgcctgaaggagcgcatccagcgccgcctccaggacatcacccagccccaccatctgctcggcctcatcgacgccgtgcagcgcctgggcgtggcctaccagttcgaggaagagatctcggacgcgctgcacggcctccattcggagaacaccgagcacgccatcaaggactcgctgcaccatacgtcgctctatttccgcctgctccgccagcatggctgcaacctgtcgtcggacatcttcaacaagttcaagaaggaaggcggcggcttcaaggcctcgctctgcgaggacgccatgggcctgctctcgctgtatgaggccgtgcgcctctcggtgaagggcgaggccatcctggaggaagcccaggtgttctcgatcgccaacctgaagatcctcatggagcgcgtggagcgcaagctcgccgaccgcatcgagcatgccctggagatcccgctctattggcgcgccccgcgtctggaggcccgctggtacatcgacgtgtatgagaaggaagacggccgcatcgacgacctgctcgacttcgcgaagctggacttcaaccgcgtgcagatgctctatcagaccgagctgaaggagctctcgatgtggtgggagctgctgggcctgcccgccaagatgggcttcttccgcgaccgcctgctcgagaaccacctcttctcgatcgccgtggtggtggagccccagtactcgcagtgccgcgtggccatcaccaaggcgatcgtgctgatgacggcgatggacgacttctatgacgtgcatggcctgccggacgagctcaaggtgttcaccgacacggtgaaccgctgggacctggagggcatcgaccagctccccgagtacatgaagctgtactatctggcgctctacaacaccacgaacgagacggcctatatcatcctgaaggagaagggcttcaacgccacgcattacctgaagaagctctgggccatgcagtcgaacgcgtatttccgcgaggcccagtggttcaactcgggctacatcccgaagttcgacgagtatctggacaacgccctcgtgtcggtgggcgccccgttcgtgctgggcctctcgtatcccatgatccagcagcagatctcgaaggaagagatcgacctgatccccgaggacctcaacctgctccgctgggcctcgatcatcttccgcctgtacgacgacctggccacctcgaaggccgagcagcagcgcggcgacgtgcccaagtcgatccagtgctatatgcatgagacgggctcgtcggaggaagtggcggccaaccatatccgcgacctgatctcggacgcgtggaaggaagtgaacgccgagtgcctgaagccgacctcgctctcgaagcactacgtgggcgtggcccccaactcggcccgctcgggcgtgctcatgtatcaccatgacttcgacggcttcgcgtcgccccatggccgcacgaacgcccacatcacgagcatcttcttcgagccggtccccctcaaggagagcatcaacctgggctga

SEQ ID NO: 32 - protein, 1048 aa, artificial
  NusA-CiCaSSy
MNKEILAVVEAVSNEKALPREKIFEALESALATATKKKYEQEIDVRVQIDRKSGDFDTFRRWLVVDEVTQPTKEITLEAARYEDESLNLGDYVEDQIESVTFDRITTQTAKQVIVQKVREAERAMVVDQFREHEGEIITGVVKKVNRDNISLDLGNNAEAVILREDMLPRENFRPGDRVRGVLYSVRPEARGAQLFVTRSKPEMLIELFRIEVPEIGEEVIEIKAAARDPGSRAKIAVKTNDKRIDPVGACVGMRGARVQAVSTELGGERIDIVLWDDNPAQFVINAMAPADVASIVVDEDKHTMDIAVEAGNLAQAIGRNGQNVRLASQLSGWELNVMTVDDLQAKHQAEAHAAIDTFTKYLDIDEDFATVLVEEGFSTLEELAYVPMKELLEIEGLDEPTVEALRERAKNALATIAQAQEESLGDNKPADDLLNLEGVDRDLAFKLAARGVCTLEDLAEQGIDDLADIEGLTDEKAGALIMAARNICWFGDEAMDSMEVRRSAIYHSTFWDIDSIRALLARRDCTAAAALSPDHHKRLKERIQRRLQDITQPHHLLGLIDAVQRLGVAYQFEEEISDALHGLHSENTEHAIKDSLHHTSLYFRLLRQHGCNLSSDIFNKFKKEGGGFKASLCEDAMGLLSLYEAVRLSVKGEAILEEAQVFSIANLKILMERVERKLADRIEHALEIPLYWRAPRLEARWYIDVYEKEDGRIDDLLDFAKLDFNRVQMLYQTELKELSMWWELLGLPAKMGFFRDRLLENHLFSIAVVVEPQYSQCRVAITKAIVLMTAMDDFYDVHGLPDELKVFTDTVNRWDLEGIDQLPEYMKLYYLALYNTTNETAYIILKEKGFNATHYLKKLWAMQSNAYFREAQWFNSGYIPKFDEYLDNALVSVGAPFVLGLSYPMIQQQISKEEIDLIPEDLNLLRWASIIFRLYDDLATSKAEQQRGDVPKSIQCYMHETGSSEEVAANHIRDLISDAWKEVNAECLKPTSLSKHYVGVAPNSARSGVLMYHHDFDGFASPHGRTNAHITSIFFEPVPLKESINLG

SEQ ID NO: 33 - protein, 594 aa, artificial
  SET-CiCaSSy
MEEASVTSTEETLTPAQEAARTRAANKARKEAELAAATAEQMDSMEVRRSAIYHSTFWDIDSIRALLARRDCTAAAALSPDHHKRLKERIQRRLQDITQPHHLLGLIDAVQRLGVAYQFEEEISDALHGLHSENTEHAIKDSLHHTSLYFRLLRQHGCNLSSDIFNKFKKEGGGFKASLCEDAMGLLSLYEAVRLSVKGEAILEEAQVFSIANLKILMERVERKLADRIEHALEIPLYWRAPRLEARWYIDVYEKEDGRIDDLLDFAKLDFNRVQMLYQTELKELSMWWELLGLPAKMGFFRDRLLENHLFSIAVVVEPQYSQCRVAITKAIVLMTAMDDFYDVHGLPDELKVFTDTVNRWDLEGIDQLPEYMKLYYLALYNTTNETAYIILKEKGFNATHYLKKLWAMQSNAYFREAQWFNSGYIPKFDEYLDNALVSVGAPFVLGLSYPMIQQQISKEEIDLIPEDLNLLRWASIIFRLYDDLATSKAEQQRGDVPKSIQCYMHETGSSEEVAANHIRDLISDAWKEVNAECLKPTSLSKHYVGVAPNSARSGVLMYHHDFDGFASPHGRTNAHITSIFFEPVPLKESINLG